European Patent Specification EP 4 081 513 B1, published November 20, 2024. Title: SUBSTITUTED QUINOLINONYL COMPOUNDS USEFUL AS T CELL ACTIVATORS. Applicant: BRISTOL-MYERS SQUIBB COMPANY. The sequence listing filed with the application follows.

SEQUENCE LISTING (6 sequences)

SEQ ID NO: 1 - DNA, 2256 bp, Homo sapiens
atggccaaggagaggggcctaataagccccagtgattttgcccagctgcaaaaatacatggaatactccaccaaaaaggtcagtgatgtcctaaagctcttcgaggatggcgagatggctaaatatgtccaaggagatgccattgggtacgagggattccagcaattcctgaaaatctatctcgaagtggataatgttcccagacacctaagcctggcactgtttcaatcctttgagactggtcactgcttaaatgagacaaatgtgacaaaagatgtggtgtgtctcaatgatgtttcctgctacttttcccttctggagggtggtcggccagaagacaagttagaattcaccttcaagctgtacgacacggacagaaatgggatcctggacagctcagaagtggacaaaattatcctacagatgatgcgagtggctgaatacctggattgggatgtgtctgagctgaggccgattcttcaggagatgatgaaagagattgactatgatggcagtggctctgtctctcaagctgagtgggtccgggctggggccaccaccgtgccactgctagtgctgctgggtctggagatgactctgaaggacgacggacagcacatgtggaggcccaagaggttccccagaccagtctactgcaatctgtgcgagtcaagcattggtcttggcaaacagggactgagctgtaacctctgtaagtacactgttcacgaccagtgtgccatgaaagccctgccttgtgaagtcagcacctatgccaagtctcggaaggacattggtgtccaatcacatgtgtgggtgcgaggaggctgtgagtccgggcgctgcgaccgctgtcagaaaaagatccggatctaccacagtctgaccgggctgcattgtgtatggtgccacctagagatccacgatgactgcctgcaagcggtgggccatgagtgtgactgtgggctgctccgggatcacatcctgcctccatcttccatctatcccagtgtcctggcctctggaccggatcgtaaaaatagcaaaacaagccagaagaccatggatgatttaaatttgagcacctctgaggctctgcggattgaccctgttcctaacacccacccacttctcgtctttgtcaatcctaagagtggcgggaagcaggggcagagggtgctctggaagttccagtatatattaaaccctcgacaggtgttcaacctcctaaaggatggtcctgagatagggctccgattattcaaggatgttcctgatagccggattttggtgtgtggtggagacggcacagtaggctggattctagagaccattgacaaagctaacttgccagttttgcctcctgttgctgtgttgcccctgggtactggaaatgatctggctcgatgcctaagatggggaggaggttatgaaggacagaatctggcaaagatcctcaaggatttagagatgagtaaagtggtacatatggatcgatggtctgtggaggtgatacctcaacaaactgaagaaaaaagtgacccagtcccctttcaaatcatcaataactacttctctattggcgtggatgcctctattgctcatcgattccacatcatgcgagagaaatatccggagaagttcaacagcagaatgaagaacaagctatggtacttcgaatttgccacatctgaatccatcttctcaacatgcaaaaagctggaggagtctttgacagttgagatctgtgggaaaccgctggatctgagcaacctgtccctagaaggcatcgcagtgctaaacatccctagcatgcatggtggctccaacctctggggtgataccaggagaccccatggggatatctatgggatcaaccaggccttaggtgctacagctaaagtcatcaccgaccctgatatcctgaaaacctgtgtaccagacctaagtgacaagagactggaagtggttgggctggagggtgcaattgagatgggccaaatctataccaagctcaagaatgctggacgtcggctggccaagtgctctgagatcaccttccacaccacaaaaacccttcccatgcaaattgacggagaaccctggatgcagacgccctgtacaatcaagatcacccacaagaaccagatgcccatgctcatgggcccacccccccgctccaccaatttctttggcttcttgagcggatcctcggagacagtgcggtttcagggacaccaccaccatcaccactga

SEQ ID NO: 2 - protein, 737 aa, Homo sapiens
MASPSDFAQLQKYMEYSTKKVSDVLKLFEDGEMAKYVQGDAIGYEGFQQFLKIYLEVDNVPRHLSLALFQSFETGHCLNETNVTKDVVCLNDVSCYFSLLEGGRPEDKLEFTFKLYDTDRNGILDSSEVDKIILQMMRVAEYLDWDVSELRPILQEMMKEIDYDGSGSVSQAEWVRAGATTVPLLVLLGLEMTLKDDGQHMWRPKRFPRPVYCNLCESSIGLGKQGLSCNLCKYTVHDQCAMKALPCEVSTYAKSRKDIGVQSHVWVRGGCESGRCDRCQKKIRIYHSLTGLHCVWCHLEIHDDCLQAVGHECDCGLLRDHILPPSSIYPSVLASGPDRKNSKTSQKTMDDLNLSTSEALRIDPVPNTHPLLVFVNPKSGGKQGQRVLWKFQYILNPRQVFNLLKDGPEIGLRLFKDVPDSRILVCGGDGTVGWILETIDKANLPVLPPVAVLPLGTGNDLARCLRWGGGYEGQNLAKILKDLEMSKVVHMDRWSVEVIPQQTEEKSDPVPFQIINNYFSIGVDASIAHRFHIMREKYPEKFNSRMKNKLWYFEFATSESIFSTCKKLEESLTVEICGKPLDLSNLSLEGIAVLNIPSMHGGSNLWGDTRRPHGDIYGINQALGATAKVITDPDILKTCVPDLSDKRLEVVGLEGAIEMGQIYTKLKNAGRRLAKCSEITFHTTKTLPMQIDGEPWMQTPCTIKITHKNQMPMLMGPPPRSGSSETVRFQGHHHHHH

SEQ ID NO: 3 - protein, 2838 aa, Homo sapiens
ATGGAGCCGCGGGACGGTAGCCCCGAGGCCCGGAGCAGCGACTCCGAGTCGGCTTCCGCCTCGTCCAGCGGCTCCGAGCGCGACGCCGGTCCCGAGCCGGACAAGGCGCCGCGGCGACTCAACAAGCGGCGCTTCCCGGGGCTGCGGCTCTTCGGGCACAGGAAAGCCATCACGAAGTCGGGCCTCCAGCACCTGGCCCCCCCTCCGCCCACCCCTGGGGCCCCGTGCAGCGAGTCAGAGCGGCAGATCCGGAGTACAGTGGACTGGAGCGAGTCAGCGACATATGGGGAGCACATCTGGTTCGAGACCAACGTGTCCGGGGACTTCTGCTACGTTGGGGAGCAGTACTGTGTAGCCAGGATGCTGCAGAAGTCAGTGTCTCGAAGAAAGTGCGCAGCCTGCAAGATTGTGGTGCACACGCCCTGCATCGAGCAGCTGGAGAAGATAAATTTCCGCTGTAAGCCGTCCTTCCGTGAATCAGGCTCCAGGAATGTCCGCGAGCCAACCTTTGTACGGCACCACTGGGTACACAGACGACGCCAGGACGGCAAGTGTCGGCACTGTGGGAAGGGATTCCAGCAGAAGTTCACCTTCCACAGCAAGGAGATTGTGGCCATCAGCTGCTCGTGGTGCAAGCAGGCATACCACAGCAAGGTGTCCTGCTTCATGCTGCAGCAGATCGAGGAGCCGTGCTCGCTGGGGGTCCACGCAGCCGTGGTCATCCCGCCCACCTGGATCCTCCGCGCCCGGAGGCCCCAGAATACTCTGAAAGCAAGCAAGAAGAAGAAGAGGGCATCCTTCAAGAGGAAGTCCAGCAAGAAAGGGCCTGAGGAGGGCCGCTGGAGACCCTTCATCATCAGGCCCACCCCCTCCCCGCTCATGAAGCCCCTGCTGGTGTTTGTGAACCCCAAGAGTGGGGGCAACCAGGGTGCAAAGATCATCCAGTCTTTCCTCTGGTATCTCAATCCCCGACAAGTCTTCGACCTGAGCCAGGGAGGGCCCAAGGAGGCGCTGGAGATGTACCGCAAAGTGCACAACCTGCGGATCCTGGCGTGCGGGGGCGACGGCACGGTGGGCTGGATCCTCTCCACCCTGGACCAGCTACGCCTGAAGCCGCCACCCCCTGTTGCCATCCTGCCCCTGGGTACTGGCAACGACTTGGCCCGAACCCTCAACTGGGGTGGGGGCTACACAGATGAGCCTGTGTCCAAGATCCTCTCCCACGTGGAGGAGGGGAACGTGGTACAGCTGGACCGCTGGGACCTCCACGCTGAGCCCAACCCCGAGGCAGGGCCTGAGGACCGAGATGAAGGCGCCACCGACCGGTTGCCCCTGGATGTCTTCAACAACTACTTCAGCCTGGGCTTTGACGCCCACGTCACCCTGGAGTTCCACGAGTCTCGAGAGGCCAACCCAGAGAAATTCAACAGCCGCTTTCGGAATAAGATGTTCTACGCCGGGACAGCTTTCTCTGACTTCCTGATGGGCAGCTCCAAGGACCTGGCCAAGCACATCCGAGTGGTGTGTGATGGAATGGACTTGACTCCCAAGATCCAGGACCTGAAACCCCAGTGTGTTGTTTTCCTGAACATCCCCAGGTACTGTGCGGGCACCATGCCCTGGGGCCACCCTGGGGAGCACCACGACTTTGAGCCCCAGCGGCATGACGACGGCTACCTCGAGGTCATTGGCTTCACCATGACGTCGTTGGCCGCGCTGCAGGTGGGCGGACACGGCGAGCGGCTGACGCAGTGTCGCGAGGTGGTGCTCACCACATCCAAGGCCATCCCGGTGCAGGTGGATGGCGAGCCCTGCAAGCTTGCAGCCTCACGCATCCGCATCGCCCTGCGCAACCAGGCCACCATGGTGCAGAAGGCCAAGCGGCGGAGCGCCGCCCCCCTGCACAGCGACCAGCAGCCGGTGCCAGAGCAGTTGCGCATCCAGGTGAGTCGCGTCAGCATGCACGACTATGAGGCCCTGCACTACGACAAGGAGCAGCTCAAGGAGGCCTCTGTGCCGCTGGGCACTGTGGTGGTCCCAGGAGACAGTGACCTAGAGCTCTGCCGTGCCCACATTGAGAGACTCCAGCAGGAGCCCGATGGTGCTGGAGCCAAGTCCCCGACATGCCAGAAACTGTCCCCCAAGTGGTGCTTCCTGGACGCCACCACTGCCAGCCGCTTCTACAGGATCGACCGAGCCCAGGAGCACCTCAACTATGTGACTGAGATCGCACAGGATGAGATTTATATCCTGGACCCTGAGCTGCTGGGGGCATCGGCCCGGCCTGACCTCCCAACCCCCACTTCCCCTCTCCCCACCTCACCCTGCTCACCCACGCCCCGGTCACTGCAAGGGGATGCTGCACCCCCTCAAGGTGAAGAGCTGATTGAGGCTGCCAAGAGGAACGACTTCTGTAAGCTCCAGGAGCTGCACCGAGCTGGGGGCGACCTCATGCACCGAGACGAGCAGAGTCGCACGCTCCTGCACCACGCAGTCAGCACTGGCAGCAAGGATGTGGTCCGCTACCTGCTGGACCACGCCCCCCCAGAGATCCTTGATGCGGTGGAGGAAAACGGGGAGACCTGTTTGCACCAAGCAGCGGCCCTGGGCCAGCGCACCATCTGCCACTACATCGTGGAGGCCGGGGCCTCGCTCATGAAGACAGACCAGCAGGGCGACACTCCCCGGCAGCGGGCTGAGAAGGCTCAGGACACCGAGCTGGCCGCCTACCTGGAGAACCGGCAGCACTACCAGATGATCCAGCGGGAGGACCAGGAGACGGCTGTGGGATCCTCGGAGACAGTGCGGTTTCAGGGACACCACCACCATCACCACTGA

SEQ ID NO: 4 - protein, 945 aa, Homo sapiens
MEPRDGSPEARSSDSESASASSSGSERDAGPEPDKAPRRLNKRRFPGLRLFGHRKAITKSGLQHLAPPPPTPGAPCSESERQIRSTVDWSESATYGEHIWFETNVSGDFCYVGEQYCVARMLQKSVSRRKCAACKIVVHTPCIEQLEKINFRCKPSFRESGSRNVREPTFVRHHWVHRRRQDGKCRHCGKGFQQKFTFHSKEIVAISCSWCKQAYHSKVSCFMLQQIEEPCSLGVHAAVVIPPTWILRARRPQNTLKASKKKKRASFKRKSSKKGPEEGRWRPFIIRPTPSPLMKPLLVFVNPKSGGNQGAKIIQSFLWYLNPRQVFDLSQGGPKEALEMYRKVHNLRILACGGDGTVGWILSTLDQLRLKPPPPVAILPLGTGNDLARTLNWGGGYTDEPVSKILSHVEEGNVVQLDRWDLHAEPNPEAGPEDRDEGATDRLPLDVFNNYFSLGFDAHVTLEFHESREANPEKFNSRFRNKMFYAGTAFSDFLMGSSKDLAKHIRVVCDGMDLTPKIQDLKPQCVVFLNIPRYCAGTMPWGHPGEHHDFEPQRHDDGYLEVIGFTMTSLAALQVGGHGERLTQCREVVLTTSKAIPVQVDGEPCKLAASRIRIALRNQATMVQKAKRRSAAPLHSDQQPVPEQLRIQVSRVSMHDYEALHYDKEQLKEASVPLGTVVVPGDSDLELCRAHIERLQQEPDGAGAKSPTCQKLSPKWCFLDATTASRFYRIDRAQEHLNYVTEIAQDEIYILDPELLGASARPDLPTPTSPLPTSPCSPTPRSLQGDAAPPQGEELIEAAKRNDFCKLQELHRAGGDLMHRDEQSRTLLHHAVSTGSKDVVRYLLDHAPPEILDAVEENGETCLHQAAALGQRTICHYIVEAGASLMKTDQQGDTPRQRAEKAQDTELAAYLENRQHYQMIQREDQETAVGSSETVRFQGHHHHHH

SEQ ID NO: 5 - protein, 2214 aa, Homo sapiens
ATGGCTTCCCCAAGCGACTTCGCCCAGCTGCAGAAGTACATGGAATACAGCACCAAGAAGGTGTCTGACGTCCTGAAGCTGTTCGAGGACGGTGAAATGGCTAAGTACGTCCAGGGCGACGCTATCGGATACGAGGGATTCCAGCAGTTCCTGAAGATCTACCTGGAAGTGGACAACGTCCCCAGGCACCTGTCACTGGCTCTGTTCCAGTCCTTCGAGACTGGCCACTGCCTGAACGAAACCAACGTCACTAAGGACGTGGTCTGCCTGAACGACGTGAGCTGCTACTTCTCTCTGCTGGAGGGTGGCAGACCAGAGGACAAGCTGGAATTCACCTTCAAGCTGTACGACACTGACCGCAACGGAATCCTGGACTCCAGCGAAGTGGACAAGATCATCCTGCAGATGATGCGTGTCGCTGAGTACCTGGACTGGGACGTGAGCGAACTGAGGCCTATCCTGCAGGAGATGATGAAGGAAATCGACTACGACGGCTCTGGATCAGTGTCCCAGGCTGAGTGGGTCCGCGCTGGTGCTACCACTGTGCCACTGCTGGTCCTGCTGGGACTGGAAATGACCCTGAAGGACGACGGTCAGCACATGTGGCGCCCAAAGCGTTTCCCCAGGCCAGTCTACTGCAACCTGTGCGAGTCTTCAATCGGTCTGGGCAAGCAGGGCCTGTCATGCAACCTGTGCAAGTACACCGTGCACGACCAGTGCGCTATGAAGGCCCTGCCCTGCGAGGTCTCAACTTACGCTAAGTCCCGTAAGGACATCGGAGTGCAGTCACACGTGTGGGTCAGGGGAGGTTGCGAATCCGGTAGATGCGACCGCTGCCAGAAGAAGATCCGTATCTACCACTCCCTGACCGGACTGCACTGCGTCTGGTGCCACCTGGAGATCCACGACGACTGCCTGCAGGCCGTGGGACACGAATGCGACTGCGGTCTGCTGCGTGACCACATCCTGCCTCCCTCCAGCATCTACCCTTCAGTCCTGGCTTCCGGTCCCGACAGGAAGAACAGCAAGACCTCTCAGAAGACTATGGACGACCTGAACCTGAGCACCTCTGAGGCCCTGCGCATCGACCCTGTGCCCAACACTCACCCACTGCTGGTGTTCGTCAACCCTAAGAGCGGCGGAAAGCAGGGTCAGAGAGTCCTGTGGAAGTTCCAGTACATCCTGAACCCACGCCAGGTGTTCAACCTGCTGAAGGACGGCCCTGAGATCGGACTGAGACTGTTCAAGGACGTGCCCGACTCTCGCATCCTCGTCTGCGGTGGCGACGGTACTGTGGGATGGATCCTGGAAACTATCGACAAGGCTAACCTGCCAGTGCTGCCACCTGTGGCTGTCCTGCCACTGGGAACCGGTAACGACCTGGCTCGTTGCCTGCGTTGGGGAGGTGGCTACGAGGGACAGAACCTGGCCAAGATCCTGAAGGACCTGGAAATGAGCAAGGTGGTCCACATGGACAGATGGTCTGTGGAGGTCATCCCACAGCAGACTGAGGAAAAGTCAGACCCAGTCCCTTTCCAGATCATCAACAACTACTTCAGCATCGGTGTGGACGCTTCTATCGCCCACAGATTCCACATCATGCGCGAGAAGTACCCTGAAAAGTTCAACTCCCGCATGAAGAACAAGCTGTGGTACTTCGAGTTCGCTACCTCAGAATCCATCTTCTCAACTTGCAAGAAGCTGGAGGAATCCCTGACCGTCGAGATCTGCGGCAAGCCTCTGGACCTGTCAAACCTGTCCCTGGAAGGCATCGCTGTGCTGAACATCCCAAGCATGCACGGAGGTTCTAACCTCTGGGGCGACACTAGGAGGCCTCACGGTGACATCTACGGCATCAACCAGGCCCTGGGAGCTACCGCCAAGGTCATCACTGACCCCGACATCCTGAAGACCTGCGTGCCAGACCTGAGCGACAAGCGTCTGGAGGTGGTCGGACTGGAGGGTGCCATCGAAATGGGCCAGATCTACACTAAGCTGAAGAACGCTGGAAGGAGACTGGCCAAGTGCTCTGAGATCACCTTCCACACCACTAAGACTCTGCCTATGCAGATCGACGGTGAACCCTGGATGCAGACCCCATGCACTATCAAGATCACCCACAAGAACCAGATGCCCATGCTGATGGGTCCTCCTCCTCGCTCTGGATCTTCAGAAACTGTGAGGTTCCAGGGCCACCACCACCACCACCACTGA

SEQ ID NO: 6 - protein, 737 aa, Homo sapiens; identical to SEQ ID NO: 2